European Patent Specification EP 3 538 552 B1, published September 13, 2023. Title: MODIFIED FAB MOLECULES. Applicant: MORPHOSYS AG. Application EP 16198591.6. The sequence listing filed with the application follows.

SEQUENCE LISTING (104 sequences)

SEQ ID NO: 1 - protein, 98 aa, Homo sapiens
ASTKGPSVFPLAPSSKSTSGGTAALGCLVKDYFPEPVTVSWNSGALTSGVHTFPAVLQSSGLYSLSSVVTVPSSSLGTQTYICNVNHKPSNTKVDKKV

SEQ ID NO: 2 - protein, 98 aa, Homo sapiens
ASTKGPSVFPLAPSSKSTSGGTAALGCLVKDYFPEPVTVSWNSGALTSGVHTFPAVLQSSGLYSLSSVVTVPSSSLGTQTYICNVNHKPSNTKVDKRV

SEQ ID NO: 3 - protein, 98 aa, Homo sapiens
ASTKGPSVFPLAPCSRSTSESTAALGCLVKDYFPEPVTVSWNSGALTSGVHTFPAVLQSSGLYSLSSVVTVPSSNFGTQTYTCNVDHKPSNTKVDKTV

SEQ ID NO: 4 - protein, 98 aa, Homo sapiens
ASTKGPSVFPLAPCSRSTSGGTAALGCLVKDYFPEPVTVSWNSGALTSGVHTFPAVLQSSGLYSLSSVVTVPSSSLGTQTYTCNVNHKPSNTKVDKRV

SEQ ID NO: 5 - protein, 98 aa, Homo sapiens
ASTKGPSVFPLAPCSRSTSESTAALGCLVKDYFPEPVTVSWNSGALTSGVHTFPAVLQSSGLYSLSSVVTVPSSSLGTKTYTCNVDHKPSNTKVDKRV

SEQ ID NO: 6 - protein, 98 aa, Artificial Sequence
  source: /note="Description of Artificial Sequence: Synthetic polypeptide"
  MOD_RES (95)..(95): Any amino acid except Cys
  MOD_RES (97)..(98): Any amino acid except Cys
ASTKGPSVFPLAPSSKSTSGGTAALGCLVKDYFPEPVTVSWNSGALTSGVHTFPAVLQSSGLYSLSSVVTVPSSSLGTQTYICNVNHKPSNTKVXKXX

SEQ ID NO: 7 - protein, 98 aa, Artificial Sequence
  source: /note="Description of Artificial Sequence: Synthetic polypeptide"
ASTKGPSVFPLAPSSKSTSGGTAALGCLVKDYFPEPVTVSWNSGALTSGVHTFPAVLQSSGLYSLSSVVTVPSSSLGTQTYICNVNHKPSNTKVDKKI

SEQ ID NO: 8 - protein, 98 aa, Artificial Sequence
  source: /note="Description of Artificial Sequence: Synthetic polypeptide"
ASTKGPSVFPLAPSSKSTSGGTAALGCLVKDYFPEPVTVSWNSGALTSGVHTFPAVLQSSGLYSLSSVVTVPSSSLGTQTYICNVNHKPSNTKVEKKV

SEQ ID NO: 9 - protein, 98 aa, Artificial Sequence
  source: /note="Description of Artificial Sequence: Synthetic polypeptide"
ASTKGPSVFPLAPSSKSTSGGTAALGCLVKDYFPEPVTVSWNSGALTSGVHTFPAVLQSSGLYSLSSVVTVPSSSLGTQTYICNVNHKPSNTKVDKGV

SEQ ID NO: 10 - protein, 98 aa, Artificial Sequence
  source: /note="Description of Artificial Sequence: Synthetic polypeptide"
ASTKGPSVFPLAPSSKSTSGGTAALGCLVKDYFPEPVTVSWNSGALTSGVHTFPAVLQSSGLYSLSSVVTVPSSSLGTQTYICNVNHKPSNTKVDKEV

SEQ ID NO: 11 - protein, 15 aa, Homo sapiens
EPKSCDKTHTCPPCP

SEQ ID NO: 12 - protein, 12 aa, Homo sapiens
ERKCCVECPPCP

SEQ ID NO: 13 - protein, 17 aa, Homo sapiens
ELKTPLGDTTHTCPRCP

SEQ ID NO: 14 - protein, 15 aa, Homo sapiens
EPKSCDTPPPCPRCP

SEQ ID NO: 15 - protein, 12 aa, Homo sapiens
ESKYGPPCPSCP

SEQ ID NO: 16 - protein, 15 aa, Rattus sp.
VPRNCGGDCKPCICT

SEQ ID NO: 17 - protein, 15 aa, Artificial Sequence
  source: /note="Description of Artificial Sequence: Synthetic peptide"
  MOD_RES (5)..(5): Any amino acid except Cys
  MOD_RES (9)..(9): Any amino acid except Cys
  MOD_RES (12)..(12): Any amino acid except Cys
VPRNXGGDXKPXICT

SEQ ID NO: 18 - protein, 15 aa, Artificial Sequence
  source: /note="Description of Artificial Sequence: Synthetic peptide"
  MOD_RES (5)..(5): Any amino acid except Cys
  MOD_RES (9)..(9): Any amino acid except Cys
  MOD_RES (14)..(14): Any amino acid except Cys
VPRNXGGDXKPCIXT

SEQ ID NO: 19 - protein, 15 aa, Artificial Sequence
  source: /note="Description of Artificial Sequence: Synthetic peptide"
  MOD_RES (5)..(5): Any amino acid except Cys
  MOD_RES (12)..(12): Any amino acid except Cys
  MOD_RES (14)..(14): Any amino acid except Cys
VPRNXGGDCKPXIXT

SEQ ID NO: 20 - protein, 15 aa, Artificial Sequence
  source: /note="Description of Artificial Sequence: Synthetic peptide"
  MOD_RES (9)..(9): Any amino acid except Cys
  MOD_RES (12)..(12): Any amino acid except Cys
  MOD_RES (14)..(14): Any amino acid except Cys
VPRNCGGDXKPXIXT

SEQ ID NO: 21 - protein, 5 aa, Rattus sp.
VPRNC

SEQ ID NO: 22 - protein, 11 aa, Rattus sp.
VPRECNPCGCT

SEQ ID NO: 23 - protein, 11 aa, Artificial Sequence
  source: /note="Description of Artificial Sequence: Synthetic peptide"
  MOD_RES (8)..(8): Any amino acid except Cys
  MOD_RES (10)..(10): Any amino acid except Cys
VPRECNPXGXT

SEQ ID NO: 24 - protein, 11 aa, Artificial Sequence
  source: /note="Description of Artificial Sequence: Synthetic peptide"
  MOD_RES (5)..(5): Any amino acid except Cys
  MOD_RES (10)..(10): Any amino acid except Cys
VPREXNPCGXT

SEQ ID NO: 25 - protein, 11 aa, Artificial Sequence
  source: /note="Description of Artificial Sequence: Synthetic peptide"
  MOD_RES (5)..(5): Any amino acid except Cys
  MOD_RES (8)..(8): Any amino acid except Cys
VPREXNPXGCT

SEQ ID NO: 26 - protein, 5 aa, Rattus sp.
VPREC

SEQ ID NO: 27 - protein, 21 aa, Rattus sp.
ERRNGGIGHKCPTCPTCHKCP

SEQ ID NO: 28 - protein, 21 aa, Artificial Sequence
  source: /note="Description of Artificial Sequence: Synthetic peptide"
  MOD_RES (14)..(14): Any amino acid except Cys
  MOD_RES (17)..(17): Any amino acid except Cys
  MOD_RES (20)..(20): Any amino acid except Cys
ERRNGGIGHKCPTXPTXHKXP

SEQ ID NO: 29 - protein, 21 aa, Artificial Sequence
  source: /note="Description of Artificial Sequence: Synthetic peptide"
  MOD_RES (11)..(11): Any amino acid except Cys
  MOD_RES (17)..(17): Any amino acid except Cys
  MOD_RES (20)..(20): Any amino acid except Cys
ERRNGGIGHKXPTCPTXHKXP

SEQ ID NO: 30 - protein, 21 aa, Artificial Sequence
  source: /note="Description of Artificial Sequence: Synthetic peptide"
  MOD_RES (11)..(11): Any amino acid except Cys
  MOD_RES (14)..(14): Any amino acid except Cys
  MOD_RES (20)..(20): Any amino acid except Cys
ERRNGGIGHKXPTXPTCHKXP

SEQ ID NO: 31 - protein, 21 aa, Artificial Sequence
  source: /note="Description of Artificial Sequence: Synthetic peptide"
  MOD_RES (11)..(11): Any amino acid except Cys
  MOD_RES (14)..(14): Any amino acid except Cys
  MOD_RES (17)..(17): Any amino acid except Cys
ERRNGGIGHKXPTXPTXHKCP

SEQ ID NO: 32 - protein, 11 aa, Rattus sp.
ERRNGGIGHKC

SEQ ID NO: 33 - protein, 11 aa, Artificial Sequence
  source: /note="Description of Artificial Sequence: Synthetic peptide"
  MOD_RES (4)..(5): Any amino acid except Cys
  source: /note="See specification as filed for detailed description of substitutions and preferred embodiments"
ERRXXGIGHKC

SEQ ID NO: 34 - protein, 11 aa, Artificial Sequence
  source: /note="Description of Artificial Sequence: Synthetic peptide"
ERRQGGIGHKC

SEQ ID NO: 35 - protein, 15 aa, Rattus sp.
EPRRPKPRPPTDICS

SEQ ID NO: 36 - protein, 14 aa, Rattus sp.
EPRRPKPRPPTDIC

SEQ ID NO: 37 - protein, 13 aa, Mus sp.
VPRDCGCKPCICT

SEQ ID NO: 38 - protein, 13 aa, Artificial Sequence
  source: /note="Description of Artificial Sequence: Synthetic peptide"
  MOD_RES (5)..(5): Any amino acid except Cys
  MOD_RES (7)..(7): Any amino acid except Cys
  MOD_RES (10)..(10): Any amino acid except Cys
VPRDXGXKPXICT

SEQ ID NO: 39 - protein, 13 aa, Artificial Sequence
  source: /note="Description of Artificial Sequence: Synthetic peptide"
  MOD_RES (7)..(7): Any amino acid except Cys
  MOD_RES (10)..(10): Any amino acid except Cys
  MOD_RES (12)..(12): Any amino acid except Cys
VPRDCGXKPXIXT

SEQ ID NO: 40 - protein, 13 aa, Artificial Sequence
  source: /note="Description of Artificial Sequence: Synthetic peptide"
  MOD_RES (5)..(5): Any amino acid except Cys
  MOD_RES (10)..(10): Any amino acid except Cys
  MOD_RES (12)..(12): Any amino acid except Cys
VPRDXGCKPXIXT

SEQ ID NO: 41 - protein, 13 aa, Artificial Sequence
  source: /note="Description of Artificial Sequence: Synthetic peptide"
  MOD_RES (5)..(5): Any amino acid except Cys
  MOD_RES (7)..(7): Any amino acid except Cys
  MOD_RES (12)..(12): Any amino acid except Cys
VPRDXGXKPCIXT

SEQ ID NO: 42 - protein, 5 aa, Mus sp.
VPRDC

SEQ ID NO: 43 - protein, 16 aa, Mus sp.
EPRGPTIKPCPPCKCP

SEQ ID NO: 44 - protein, 16 aa, Artificial Sequence
  source: /note="Description of Artificial Sequence: Synthetic peptide"
  MOD_RES (13)..(13): Any amino acid except Cys
  MOD_RES (15)..(15): Any amino acid except Cys
EPRGPTIKPCPPXKXP

SEQ ID NO: 45 - protein, 16 aa, Artificial Sequence
  source: /note="Description of Artificial Sequence: Synthetic peptide"
  MOD_RES (10)..(10): Any amino acid except Cys
  MOD_RES (15)..(15): Any amino acid except Cys
EPRGPTIKPXPPCKXP

SEQ ID NO: 46 - protein, 16 aa, Artificial Sequence
  source: /note="Description of Artificial Sequence: Synthetic peptide"
  MOD_RES (10)..(10): Any amino acid except Cys
  MOD_RES (13)..(13): Any amino acid except Cys
EPRGPTIKPXPPXKCP

SEQ ID NO: 47 - protein, 10 aa, Mus sp.
EPRGPTIKPC

SEQ ID NO: 48 - protein, 22 aa, Mus sp.
EPSGPISTINPCPPCKECHKCP

SEQ ID NO: 49 - protein, 22 aa, Artificial Sequence
  source: /note="Description of Artificial Sequence: Synthetic peptide"
  MOD_RES (15)..(15): Any amino acid except Cys
  MOD_RES (18)..(18): Any amino acid except Cys
  MOD_RES (21)..(21): Any amino acid except Cys
EPSGPISTINPCPPXKEXHKXP

SEQ ID NO: 50 - protein, 22 aa, Artificial Sequence
  source: /note="Description of Artificial Sequence: Synthetic peptide"
  MOD_RES (12)..(12): Any amino acid except Cys
  MOD_RES (18)..(18): Any amino acid except Cys
  MOD_RES (21)..(21): Any amino acid except Cys
EPSGPISTINPXPPCKEXHKXP

SEQ ID NO: 51 - protein, 22 aa, Artificial Sequence
  source: /note="Description of Artificial Sequence: Synthetic peptide"
  MOD_RES (12)..(12): Any amino acid except Cys
  MOD_RES (15)..(15): Any amino acid except Cys
  MOD_RES (21)..(21): Any amino acid except Cys
EPSGPISTINPXPPXKECHKXP

SEQ ID NO: 52 - protein, 22 aa, Artificial Sequence
  source: /note="Description of Artificial Sequence: Synthetic peptide"
  MOD_RES (12)..(12): Any amino acid except Cys
  MOD_RES (15)..(15): Any amino acid except Cys
  MOD_RES (18)..(18): Any amino acid except Cys
EPSGPISTINPXPPXKEXHKCP

SEQ ID NO: 53 - protein, 12 aa, Mus sp.
EPSGPISTINPC

SEQ ID NO: 54 - protein, 21 aa, Mus sp.
EPRVPITQNPCPPLKECPPCA

SEQ ID NO: 55 - protein, 21 aa, Artificial Sequence
  source: /note="Description of Artificial Sequence: Synthetic peptide"
  MOD_RES (17)..(17): Any amino acid except Cys
  MOD_RES (20)..(20): Any amino acid except Cys
EPRVPITQNPCPPLKEXPPXA

SEQ ID NO: 56 - protein, 21 aa, Artificial Sequence
  source: /note="Description of Artificial Sequence: Synthetic peptide"
  MOD_RES (11)..(11): Any amino acid except Cys
  MOD_RES (20)..(20): Any amino acid except Cys
EPRVPITQNPXPPLKECPPXA

SEQ ID NO: 57 - protein, 21 aa, Artificial Sequence
  source: /note="Description of Artificial Sequence: Synthetic peptide"
  MOD_RES (11)..(11): Any amino acid except Cys
  MOD_RES (17)..(17): Any amino acid except Cys
EPRVPITQNPXPPLKEXPPCA

SEQ ID NO: 58 - protein, 11 aa, Mus sp.
EPRVPITQNPC

SEQ ID NO: 59 - protein, 16 aa, Mus sp.
EPRIPKPSTPPGSSCP

SEQ ID NO: 60 - protein, 15 aa, Mus sp.
EPRIPKPSTPPGSSC

SEQ ID NO: 61 - protein, 5 aa, Homo sapiens
PKSCD

SEQ ID NO: 62 - protein, 5 aa, Homo sapiens
KSCDK

SEQ ID NO: 63 - protein, 5 aa, Homo sapiens
SCDKT

SEQ ID NO: 64 - protein, 5 aa, Homo sapiens
DKTHT

SEQ ID NO: 65 - protein, 5 aa, Homo sapiens
KTHTC

SEQ ID NO: 66 - protein, 5 aa, Homo sapiens
THTCP

SEQ ID NO: 67 - protein, 5 aa, Homo sapiens
HTCPP

SEQ ID NO: 68 - protein, 5 aa, Homo sapiens
TCPPC

SEQ ID NO: 69 - protein, 5 aa, Homo sapiens
CPPCP

SEQ ID NO: 70 - protein, 103 aa, Artificial Sequence
  source: /note="Description of Artificial Sequence: Synthetic polypeptide"
ASTKGPSVFPLAPSSKSTSGGTAALGCLVKDYFPEPVTVSWNSGALTSGVHTFPAVLQSSGLYSLSSVVTVPSSSLGTQTYICNVNHKPSNTKVDKKIVPREC

SEQ ID NO: 71 - protein, 109 aa, Artificial Sequence
  source: /note="Description of Artificial Sequence: Synthetic polypeptide"
ASTKGPSVFPLAPSSKSTSGGTAALGCLVKDYFPEPVTVSWNSGALTSGVHTFPAVLQSSGLYSLSSVVTVPSSSLGTQTYICNVNHKPSNTKVDKKVERRNGGIGHKC

SEQ ID NO: 72 - protein, 109 aa, Artificial Sequence
  source: /note="Description of Artificial Sequence: Synthetic polypeptide"
ASTKGPSVFPLAPSSKSTSGGTAALGCLVKDYFPEPVTVSWNSGALTSGVHTFPAVLQSSGLYSLSSVVTVPSSSLGTQTYICNVNHKPSNTKVEKKVERRNGGIGHKC

SEQ ID NO: 73 - protein, 109 aa, Artificial Sequence
  source: /note="Description of Artificial Sequence: Synthetic polypeptide"
ASTKGPSVFPLAPSSKSTSGGTAALGCLVKDYFPEPVTVSWNSGALTSGVHTFPAVLQSSGLYSLSSVVTVPSSSLGTQTYICNVNHKPSNTKVDKGVERRNGGIGHKC

SEQ ID NO: 74 - protein, 109 aa, Artificial Sequence
  source: /note="Description of Artificial Sequence: Synthetic polypeptide"
ASTKGPSVFPLAPSSKSTSGGTAALGCLVKDYFPEPVTVSWNSGALTSGVHTFPAVLQSSGLYSLSSVVTVPSSSLGTQTYICNVNHKPSNTKVDKEVERRNGGIGHKC

SEQ ID NO: 75 - protein, 109 aa, Artificial Sequence
  source: /note="Description of Artificial Sequence: Synthetic polypeptide"
ASTKGPSVFPLAPSSKSTSGGTAALGCLVKDYFPEPVTVSWNSGALTSGVHTFPAVLQSSGLYSLSSVVTVPSSSLGTQTYICNVNHKPSNTKVDKKVEERNGGIGHKC

SEQ ID NO: 76 - protein, 109 aa, Artificial Sequence
  source: /note="Description of Artificial Sequence: Synthetic polypeptide"
ASTKGPSVFPLAPSSKSTSGGTAALGCLVKDYFPEPVTVSWNSGALTSGVHTFPAVLQSSGLYSLSSVVTVPSSSLGTQTYICNVNHKPSNTKVDKEVERRQGGIGHKC

SEQ ID NO: 77 - protein, 5 aa, Homo sapiens
CDKTH

SEQ ID NO: 78 - protein, 8 aa, Unknown
  source: /note="Description of Unknown: non-rodent hinge region peptide"
EPKSCDKT

SEQ ID NO: 79 - protein, 10 aa, Unknown
  source: /note="Description of Unknown: non-rodent hinge region peptide"
EPKSCDKTHT

SEQ ID NO: 80 - protein, 9 aa, Unknown
  source: /note="Description of Unknown: non-rodent hinge region peptide"
EPKSCDKTH

SEQ ID NO: 81 - protein, 7 aa, Unknown
  source: /note="Description of Unknown: non-rodent hinge region peptide"
EPKSCDK

SEQ ID NO: 82 - protein, 6 aa, Unknown
  source: /note="Description of Unknown: non-rodent hinge region peptide"
EPKSCD

SEQ ID NO: 83 - protein, 4 aa, Unknown
  source: /note="Description of Unknown: non-rodent hinge region peptide"
EPKS

SEQ ID NO: 84 - protein, 3 aa, Unknown
  source: /note="Description of Unknown: non-rodent hinge region peptide"
EPK

SEQ ID NO: 85 - protein, 2 aa, Unknown
  source: /note="Description of Unknown: non-rodent hinge region peptide"
EP

SEQ ID NO: 86 - protein, 4 aa, Homo sapiens
DKKV

SEQ ID NO: 87 - protein, 4 aa, Homo sapiens
DKRV

SEQ ID NO: 88 - protein, 4 aa, Artificial Sequence
  source: /note="Description of Artificial Sequence: Synthetic peptide"
EKKV

SEQ ID NO: 89 - protein, 4 aa, Artificial Sequence
  source: /note="Description of Artificial Sequence: Synthetic peptide"
DKKI

SEQ ID NO: 90 - protein, 4 aa, Artificial Sequence
  source: /note="Description of Artificial Sequence: Synthetic peptide"
DKGV

SEQ ID NO: 91 - protein, 4 aa, Artificial Sequence
  source: /note="Description of Artificial Sequence: Synthetic peptide"
DKEV

SEQ ID NO: 92 - protein, 4 aa, Artificial Sequence
  source: /note="Description of Artificial Sequence: Synthetic peptide"
  MOD_RES (1)..(1): Any amino acid except Cys
  MOD_RES (3)..(4): Any amino acid except Cys
XKXX

SEQ ID NO: 93 - protein, 11 aa, Artificial Sequence
  source: /note="Description of Artificial Sequence: Synthetic peptide"
EERNGGIGHKC

SEQ ID NO: 94 - protein, 5 aa, Homo sapiens
EPKSC

SEQ ID NO: 95 - protein, 11 aa, Homo sapiens
KVDKKVEPKSC

SEQ ID NO: 96 - protein, 11 aa, Homo sapiens
KVDKRVEPKSC

SEQ ID NO: 97 - protein, 11 aa, Artificial Sequence
  source: /note="Description of Artificial Sequence: Synthetic peptide"
KVDKKIVPREC

SEQ ID NO: 98 - protein, 17 aa, Artificial Sequence
  source: /note="Description of Artificial Sequence: Synthetic peptide"
KVDKKVERRNGGIGHKC

SEQ ID NO: 99 - protein, 17 aa, Artificial Sequence
  source: /note="Description of Artificial Sequence: Synthetic peptide"
KVEKKVERRNGGIGHKC

SEQ ID NO: 100 - protein, 17 aa, Artificial Sequence
  source: /note="Description of Artificial Sequence: Synthetic peptide"
KVDKGVERRNGGIGHKC

SEQ ID NO: 101 - protein, 17 aa, Artificial Sequence
  source: /note="Description of Artificial Sequence: Synthetic peptide"
KVDKEVERRNGGIGHKC

SEQ ID NO: 102 - protein, 17 aa, Artificial Sequence
  source: /note="Description of Artificial Sequence: Synthetic peptide"
KVDKKVEERNGGIGHKC

SEQ ID NO: 103 - protein, 17 aa, Artificial Sequence
  source: /note="Description of Artificial Sequence: Synthetic peptide"
KVDKEVERRQGGIGHKC

SEQ ID NO: 104 - protein, 61 aa, Homo sapiens
ASTKGPSVFPLAPSSKSTSGGTAALGCLVKDYFPEPVTVSWNSGALTSGVHTFPAVLQSSG